European Patent Specification EP 3 741 873 B1, published December 6, 2023. Title: Method for Identifying the Red Feather Causative Mutation Genotypes of White Leghorn Chickens and Breeding of Commercial Strains of Red Feather Pink-Shell Laying Hens. Applicant: Beijing Huadu Yukou Poultry Industry Co., Ltd. The sequence listing filed with the application follows.

SEQUENCE LISTING (3 sequences)

SEQ ID NO: 1 - DNA, 288 bp, Artificial sequence
gccgccatcctcaagaacaggaatctgcactcgcccatgtactacttcatctgctgcctggccgtctccgacatgctggtgagcgtcagcaacctggccgagacgctcttcatgctgctgatggagcacggcgtgctggtgatccgcgccagcatcgtccgccacatggacaatgtcatcgacatgctcatctgcagctccgtcgtgtcctccctctccttcctgggggtcatcgccgtggaccgctacatcacgatcttctatgcgctgcgtttttttttttttttt

SEQ ID NO: 2 - DNA, 19 bp, Artificial sequence
gccgccatcctcaagaaca

SEQ ID NO: 3 - DNA, 34 bp, Artificial sequence
aaaaaaaaaaaaaaacgcagcgcatagaagatcg